European Patent Application EP 4 435 099 A1, published September 25, 2024. Title: LOW GLYCOSYLATED KALLIKREIN I AND POLYETHYLENE GLYCOL MODIFIED PRODUCT THEREOF AND PHARMACEUTICAL APPLICATIONS THEREOF. Applicant: ZonHon Biopharma Institute Inc. Application EP. The sequence listing filed with the application follows.

SEQUENCE LISTING (6 sequences)

SEQ ID NO: 1 - protein, 238 aa, synthetic construct [sequence omitted]

SEQ ID NO: 2 - DNA, 789 bp, synthetic construct
  source 1..789: mol_type = other DNA
atgtggttcctggtgctgtgcctggccctgagcctgggcggcaccggcgccgccccccctatccagtccaggatcgtcgggggttgggagtgtgaacagcatagtcagccctggcaggccgctctgtaccacttctccacctttcagtgcggcggaatcctggtgcacaggcagtgggtcctgacagcagcccattgtattagcgataactatcagctgtggctgggccggcataacctgttcgacgatgagaataccgcccagtttgtgcacgtctcagaatccttcccccatcctggcttcaacatgagtctgctggagaatcacaccaggcaggctgacgaagattactcacatgacctgatgctgctgcgactgacagagccagcagacactatcaccgatgctgtgaaggtggtcgagctgcccacacaggaacctgaagtgggctctacttgcctggcaagcggatggggttctatcgagcctgaaaacttcagttttccagacgatctgcagtgcgtggacctgaagattctgcctaatgatgagtgtaagaaagctcacgtccagaaagtgactgattttatgctgtgcgtggggcatctggagggaggcaaggacacctgcgtcggcgactccggaggacctctgatgtgtgacggggtgctgcagggtgtcactagctggggctacgtgccatgtggaaccccaaataagccctccgtggccgtcagagtgctgagctatgtgaaatggatcgaggacaccattgctgaaaacagttga

SEQ ID NO: 3 - protein, 238 aa, synthetic construct
IVGGWECEQHSQPWQAALYHFSTFQCGGILVHRQWVLTAAHCISDNYQLWLGRHNLFDDENTAQFVHVSESFPHPGFNMSLLENHTRQADEDYSHDLMLLRLTEPADTITDAVKVVELPTQEPEVGSTCLASGWGSIEPEQFSFPDDLQCVDLKILPNDECKKAHVQKVTDFMLCVGHLEGGKDTCVGDSGGPLMCDGVLQGVTSWGYVPCGTPNKPSVAVRVLSYVKWIEDTIAENS

SEQ ID NO: 4 - protein, 238 aa, synthetic construct
IVGGWECEQHSQPWQAALYHFSTFQCGGILVHRQWVLTAAHCISDNYQLWLGRHNLFDDENTAQFVHVSESFPHPGFNMSLLENHTRQADEDYSHDLMLLRLTEPADTITDAVKVVELPTQEPEVGSTCLASGWGSIEPEDFSFPDDLQCVDLKILPNDECKKAHVQKVTDFMLCVGHLEGGKDTCVGDSGGPLMCDGVLQGVTSWGYVPCGTPNKPSVAVRVLSYVKWIEDTIAENS

SEQ ID NO: 5 - protein, 238 aa, synthetic construct
IVGGWECEQHSQPWQAALYHFSTFQCGGILVHRQWVLTAAHCISDNYQLWLGRHNLFDDENTAQFVHVSESFPHPGFNMSLLENHTRQADEDYSHDLMLLRLTEPADTITDAVKVVELPTQEPEVGSTCLASGWGSIEPERFSFPDDLQCVDLKILPNDECKKAHVQKVTDFMLCVGHLEGGKDTCVGDSGGPLMCDGVLQGVTSWGYVPCGTPNKPSVAVRVLSYVKWIEDTIAENS

SEQ ID NO: 6 - protein, 238 aa, synthetic construct
IVGGWECEQHSQPWQAALYHFSTFQCGGILVHRQWVLTAAHCISDNYQLWLGRHNLFDDENTAQFVHVSESFPHPGFNMSLLENHTRQADEDYSHDLMLLRLTEPADTITDAVKVVELPTQEPEVGSTCLASGWGSIEPEAFSFPDDLQCVDLKILPNDECKKAHVQKVTDFMLCVGHLEGGKDTCVGDSGGPLMCDGVLQGVTSWGYVPCGTPNKPSVAVRVLSYVKWIEDTIAENS